European Patent Application EP 4 578 939 A1, published July 2, 2025. Title: MYCOBACTERIUM SP. BASED ON VARIOUS CARBON-NITROGEN METABOLIC PATHWAYS, METHOD FOR ISOLATING SAME, AND USE THEREOF. Applicant: PENG Guanghao. Application WO. The sequence listing filed with the application follows.

SEQUENCE LISTING (10 sequences)

SEQ ID NO: 1 - RNA, 1379 nt, Mycobacterium sp.
  source 1..1379: mol_type = rRNA
cggctccctcccacaaggggttaggccaccggcttcgggtgttaccgacttcatgacgtgacgggcggtgtgtacaaggcccgggaacgtattcaccgcagcgtgctgatctgcgattactagcgactccgacttcacggggtcgagttgcagaccccgatccgaactgagaccggctttgaaaggattcgctccacctcacggcatcgcagccctttgtaccggccattgtagcatgtgtgaagcccgagttgaccccggcagtctctcacgagtccccgccactggacataaggggcatgatgacttgacgtcatccccaccttacgcgctggcaacataagataagggttgcgctcgttgcgggactaacccaacatctcacgacacgagctgacgacagccatgcaccacctgcacacaggccacaagggaatacctatctctaggcacgtcctgtgcatgtcaaacccaggtaaggttcttcgcgttgcatcgaattaatccacatgctccgccgcttgtgcgggcccccgtcaatttctttgagttttagccttgcggccgtactccccaggcggggtacttaatgcgttagctacggcacggatcccaaggaaggaaacccacacctagtacccaccgtttacggcgtggactaccagggtatctaatcctgttcgctccccacgctttcgctcctcagcgtcagttacgcccagagacccgccttcgccaccggtgttcctcctgatatctgcgcattccaccgctacaccaggaattccagtctcccctgcagtactccagtctgcccgtatcgcccgcacgcccacagttgagctgtgagttttcacgaacaacgcgacaaaccacctacgagctctttacgcccagtaattccggacaacgctcggaccctacgtattaccgcggctgctggcacgtagttggccggtccttcttctccaggtaccgtcacttgcgcttcgtccctggcgaaagaggtttacaacccgaaggccgtcatccctcacgcggcgtcgcgcatcaggcttgcgcccattgtgcaatattccccactgctgcctcccgtaggagtctgggccgtatctcagtcccagtgtggccggtcaccctctcaggccggctacccgtcgtcgccttggtgagccgtaacctcaccaacaagctgataggccgcgggcccatcccacaccgcaaaagctttccccaaccagaccatgcagccagaagggtgtattcggtattagacccagtttcccaggcttatcccaaagtgcagggcagatcacccacgtgttactcacccgttcgccactcgagtaccccgaagggcctttccgttcgactgcatg

SEQ ID NO: 2 - RNA, 1281 nt, Mycobacterium sp.
  source 1..1281: mol_type = rRNA
ggctccctcccacaaggggttaggccaccggcttcgggtgttaccgactttcatgacgtgacgggcggtgtgtacaaggcccgggaacgtattcaccgcagcgttgctgatctgcgattactagcgactccgacttcacggggtcgagttgcagaccccgatccgaactgagaccggctttgaaaggattcgctccacctcacggcatcgcagcccttgtaccggccattgtagcatgtgtgaagccctggacataaggggcatgatgacttgacgtcatccccaccttcctccgagttgagtctcacgagtccccgccattacgcgctggcaacataagataagggttgcgctcgttgcgggacttaacccaacacacgagctgacgacagccatgcaccacctgcacacaggccacaagggaatacctatctctaggcacgtcctgtgcataggtaaggttcttcgcgttgcatcgaattaatccacatgctccgccgcttgtgcgggcccccgtcaatcttgcggccgtactccccaggcggggtacttaatgcgttagctacggcacggatcccaaggaaggaaacccaaccgtttacggcgtggactaccagggtatctaatcctgttcgctccccacgctttcgctcctcagcgtcagtagagacccgccttcgccaccggtgttcctcctgatatctgcgcattccaccgctacaccaggaattccagtctcccagtactccagtctgcccgtatcgcccgcacgcccacagttgagctgtgagttttcacgaacaacgcgacaaacccgcccagtaattccggacaacgctcggaccctacgtattaccgcggctgctggcacgtagttggccggtcggtaccgtcacttgcgttcgtccctggcgaaagaggtttacaacccgaaggccgtcatccctcacgcggcgtaggcttgcgcccattgtgcaatattccccactgctgcctcccgtaggagtctgggccgtatctcagtcccagtgtggccggtcaccctctcaggccggcacccgtcgtcgccttggtgagccgtaacctcaccaacaagctgataggccgcgggcccatcccacaccgcaaagctttccccaaccagaccatgcagccagaagggtgtattcggtattagacccagtttcccaggcttatcccaaagtgcagggcagatcacccacgtgttactcacccgttcgccactcgagtaccccgaagggcctttccgttcgacttgca

SEQ ID NO: 3 - DNA, 20 bp, synthetic construct
  source 1..20: mol_type = other DNA
tgcgayccsaargcbgactc

SEQ ID NO: 4 - DNA, 20 bp, synthetic construct
  source 1..20: mol_type = other DNA
atsgccatcatytcrccgga

SEQ ID NO: 5 - DNA, 25 bp, synthetic construct
  source 1..25: mol_type = other DNA
acccgcctgatcctgcacgccaagg

SEQ ID NO: 6 - DNA, 26 bp, synthetic construct
  source 1..26: mol_type = other DNA
acgatgtagatttcctgggccttgtt

SEQ ID NO: 7 - DNA, 26 bp, synthetic construct
  source 1..26: mol_type = other DNA
aaaggyggwatcggyaartccaccac

SEQ ID NO: 8 - DNA, 26 bp, synthetic construct
  source 1..26: mol_type = other DNA
ttgttsgcsgcrtacatsgccatcat

SEQ ID NO: 9 - DNA, 20 bp, synthetic construct
  source 1..20: mol_type = other DNA
cgmtgttcntcgacagccag

SEQ ID NO: 10 - DNA, 21 bp, synthetic construct
  source 1..21: mol_type = other DNA
catgtgcagdgchtggcagaa